European Patent Specification EP 3 019 596 B1, published July 5, 2023. Title: COMPOSITIONS AND METHODS FOR REPROGRAMING NON-PLURIPOTENT CELLS INTO PLURIPOTENT STEM CELLS. Applicant: Grandhope Biotech Co. Ltd Hongkui, Deng Zhao, Yang Hou, Pingping Li, Yanqin Zhang, Xu Liu, Chun Guan, Jingyang Li, Honggang. The sequence listing filed with the application follows.

SEQUENCE LISTING (63 sequences)

SEQ ID NO: 1 - DNA, 35 bp, Artificial Sequence
  Synthetic forward primer for Sall4 (plasmid construction)
actcgagccaccatgtcgaggcgcaagcaggcgaa

SEQ ID NO: 2 - DNA, 35 bp, Artificial Sequence
  Synthetic reverse primer for Sall4 (plasmid construction)
gcaattgttagctgacagcaatcttattttcctcc

SEQ ID NO: 3 - DNA, 22 bp, Artificial Sequence
  Synthetic forward primer for Sox2 (qRT-PCR)
cgggaagcgtgtacttatcctt

SEQ ID NO: 4 - DNA, 21 bp, Artificial Sequence
  Synthetic reverse primer for Sox2 (qRT-PCR)
gcggagtggaaacttttgtcc

SEQ ID NO: 5 - DNA, 22 bp, Artificial Sequence
  Synthetic forward primer for Klf4 (qRT-PCR)
ttgcggtagtgcctggtcagtt

SEQ ID NO: 6 - DNA, 22 bp, Artificial Sequence
  Synthetic reverse  primer for Klf4 (qRT-PCR)
ctatgcaggctgtggcaaaacc

SEQ ID NO: 7 - DNA, 19 bp, Artificial Sequence
  Synthetic forward  primer for Oct4 (qRT-PCR)
cagggctttcatgtcctgg

SEQ ID NO: 8 - DNA, 20 bp, Artificial Sequence
  Synthetic reverse primer for Oct4 (qRT-PCR)
agttggcgtggagactttgc

SEQ ID NO: 9 - DNA, 24 bp, Artificial Sequence
  Synthetic forward primer for Gata4 (qRT-PCR)
gagctggcctgcgatgtctgagtg

SEQ ID NO: 10 - DNA, 24 bp, Artificial Sequence
  Synthetic reverse primer for Gata4 (qRT-PCR)
aaacggaagcccaagaacctgaat

SEQ ID NO: 11 - DNA, 20 bp, Artificial Sequence
  Synthetic forward  primer for Gata6 (qRT-PCR)
tgaggtggtcgcttgtgtag

SEQ ID NO: 12 - DNA, 20 bp, Artificial Sequence
  Synthetic reverse  primer for Gata6 (qRT-PCR)
atggcgtagaaatgctgagg

SEQ ID NO: 13 - DNA, 21 bp, Artificial Sequence
  Synthetic forward primer for Sox17 (qRT-PCR)
gtcaacgccttccaagacttg

SEQ ID NO: 14 - DNA, 21 bp, Artificial Sequence
  Synthetic reverse primer for Sox17 (qRT-PCR)
gtaaaggtgaaaggcgaggtg

SEQ ID NO: 15 - DNA, 19 bp, Artificial Sequence
  Synthetic forward primer for Esrrb (qRT-PCR)
gtggctgagggcatcaatg

SEQ ID NO: 16 - DNA, 21 bp, Artificial Sequence
  Synthetic reverse primer for Esrrb (qRT-PCR)
aaccgaatgtcgtccgaagac

SEQ ID NO: 17 - DNA, 21 bp, Artificial Sequence
  Synthetic forward primer for Sall4 (qRT-PCR)
tggcagacgagaagttctttc

SEQ ID NO: 18 - DNA, 22 bp, Artificial Sequence
  Synthetic reverse primer for Sall4 (qRT-PCR)
tccaacatttatccgagcacag

SEQ ID NO: 19 - DNA, 21 bp, Artificial Sequence
  Synthetic forward primer for Lin28a (qRT-PCR)
ccgcagttgtagcacctgtct

SEQ ID NO: 20 - DNA, 22 bp, Artificial Sequence
  Synthetic reverse primer for Lin28a (qRT-PCR)
gaagaacatgcagaagcgaaga

SEQ ID NO: 21 - DNA, 21 bp, Artificial Sequence
  Synthetic forward primer for Dppa2 (qRT-PCR)
gcgtagcgtagtctgtgtttg

SEQ ID NO: 22 - DNA, 22 bp, Artificial Sequence
  Synthetic reverse primer for Dppa2 (qRT-PCR)
tcaacgagaaccaatctgagga

SEQ ID NO: 23 - DNA, 21 bp, Artificial Sequence
  Synthetic forward primer for Nanog (qRT-PCR)
agttatggagcggagcagcat

SEQ ID NO: 24 - DNA, 18 bp, Artificial Sequence
  Synthetic reverse primer for Nanog (qRT-PCR)
aggcctggaccgctcagt

SEQ ID NO: 25 - DNA, 18 bp, Artificial Sequence
  Synthetic forward primer for Oct4 (genomic PCR)
gaaggatgtggtccgagt

SEQ ID NO: 26 - DNA, 20 bp, Artificial Sequence
  Synthetic reverse primer for Oct4 (genomic PCR)
gcagcgtatccacatagcgt

SEQ ID NO: 27 - DNA, 18 bp, Artificial Sequence
  Synthetic forward primer for Sox2 (genomic PCR)
catgggttcggtggtcaa

SEQ ID NO: 28 - DNA, 20 bp, Artificial Sequence
  Synthetic reverse primer for Sox2 (genomic PCR)
gcagcgtatccacatagcgt

SEQ ID NO: 29 - DNA, 18 bp, Artificial Sequence
  Synthetic forward primer for Klf4 (genomic PCR)
accactgtgactgggacg

SEQ ID NO: 30 - DNA, 20 bp, Artificial Sequence
  Synthetic reverse primer for Klf4 (genomic PCR)
gcagcgtatccacatagcgt

SEQ ID NO: 31 - DNA, 20 bp, Artificial Sequence
  Synthetic forward primer for c-Myc (genomic PCR)
tacatcctgtccgtccaagc

SEQ ID NO: 32 - DNA, 20 bp, Artificial Sequence
  Synthetic reverse primer for c-Myc (genomic PCR)
gcagcgtatccacatagcgt

SEQ ID NO: 33 - DNA, 19 bp, Artificial Sequence
  Synthetic forward primer for hOct4 (genomic PCR)
acctccatagaagacaccg

SEQ ID NO: 34 - DNA, 18 bp, Artificial Sequence
  Synthetic reverse primer for hOct4 (genomic PCR)
tagccccactccaacctg

SEQ ID NO: 35 - DNA, 19 bp, Artificial Sequence
  Synthetic forward primer for hSox2 (genomic PCR)
acctccatagaagacaccg

SEQ ID NO: 36 - DNA, 22 bp, Artificial Sequence
  Synthetic reverse primer for hSox2 (genomic PCR)
ctccgacaaaagtttccactcg

SEQ ID NO: 37 - DNA, 19 bp, Artificial Sequence
  Synthetic foerward primer for hKlf4 (genomic PCR)
acctccatagaagacaccg

SEQ ID NO: 38 - DNA, 18 bp, Artificial Sequence
  Synthetic reverse primer for hKLF4 (genomic PCR)
gaagaggaggctgacgct

SEQ ID NO: 39 - DNA, 19 bp, Artificial Sequence
  Synthetic forward primer for hcMyc (genomic PCR)
acctccatagaagacaccg

SEQ ID NO: 40 - DNA, 18 bp, Artificial Sequence
  Synthetic reverse primer for hcMyc (genomic PCR)
gggtcgcagatgaaactc

SEQ ID NO: 41 - DNA, 22 bp, Artificial Sequence
  Synthetic forward primer for Oct4 (bisulfite genomic sequencing)
ggagtggttttagaaataattg

SEQ ID NO: 42 - DNA, 23 bp, Artificial Sequence
  Synthetic reverse primer for Oct4 (bisulfite genomic sequencing)
tccaaccctactaacccatcacc

SEQ ID NO: 43 - DNA, 30 bp, Artificial Sequence
  Synthetic forward primer for Nanog (bisulfite genomic sequencing)
gattttgtaggtgggattaattgtgaattt

SEQ ID NO: 44 - DNA, 30 bp, Artificial Sequence
  Synthetic reverse primer for Nanog (bisulfite genomic sequencing)
accaaaaaaacccacactcatatcaatata

SEQ ID NO: 45 - DNA, 20 bp, Artificial Sequence
  Synthetic forward primer for Oct4 (chromatin immunoprecipitation)
ctgtaaggacaggccgagag

SEQ ID NO: 46 - DNA, 20 bp, Artificial Sequence
  Synthetic reverse primer for Oct4 (chromatin immunoprecipitation)
caggaggccttcattttcaa

SEQ ID NO: 47 - DNA, 19 bp, Artificial Sequence
  Synthetic forward primer for Nanog (chromatin immunoprecipitation)
ctatcgccttgagccgttg

SEQ ID NO: 48 - DNA, 26 bp, Artificial Sequence
  Synthetic reverse primer for Nanog (chromatin immunoprecipitation)
aactcagtgtctagaaggaaagatca

SEQ ID NO: 49 - DNA, 21 bp, Artificial Sequence
  Synthetic forward primer for Sox2 (chromatin immunoprecipitation)
tttattcagttcccagtccaa

SEQ ID NO: 50 - DNA, 22 bp, Artificial Sequence
  Synthetic reverse primer for Sox2 (chromatin immunoprecipitation)
ttattcctatgtgtgagcaaga

SEQ ID NO: 51 - DNA, 19 bp, Artificial Sequence
  Synthetic forward primer for OG (For OG (Oct4 promoter-driven GFP) cassette)
aaccactacctgagcaccc

SEQ ID NO: 52 - DNA, 20 bp, Artificial Sequence
  Synthetic reverse primer for OG (For OG (Oct4 promoter-driven GFP) cassette)
acctctacaaatgtggtatg

SEQ ID NO: 53 - DNA, 58 bp, Artificial Sequence
  Synthetic Sall4 ShRNA 1 sequence
ccggcagcccacctttgtcaaagttctcgagaactttgacaaaggtgggctgtttttg

SEQ ID NO: 54 - DNA, 58 bp, Artificial Sequence
  Synthetic Sall4 ShRNA 2 sequence
ccgggcccacctttgtcaaagttgactcgagtcaactttgacaaaggtgggctttttg

SEQ ID NO: 55 - DNA, 58 bp, Artificial Sequence
  Synthetic Gata4 ShRNA 1 sequence
ccggagcccaagaacctgaataaatctcgagatttattcaggttcttgggcttttttg

SEQ ID NO: 56 - DNA, 58 bp, Artificial Sequence
  Synthetic Gata4 ShRNA 2 sequence
ccggcatctcctgtcactcagacatctcgagatgtctgagtgacaggagatgtttttg

SEQ ID NO: 57 - DNA, 58 bp, Artificial Sequence
  Synthetic Gata6 ShRNA 1 sequence
ccggccactaccttatggcgtagaactcgagttctacgccataaggtagtggtttttg

SEQ ID NO: 58 - DNA, 58 bp, Artificial Sequence
  Synthetic Gata6 ShRNA 2 sequence
ccggcctcgaccacttgctatgaaactcgagtttcatagcaagtggtcgaggtttttg

SEQ ID NO: 59 - DNA, 58 bp, Artificial Sequence
  Synthetic Sox17 ShRNA 1 sequence
ccggcccacaatcactgtccagtttctcgagaaactggacagtgattgtgggtttttg

SEQ ID NO: 60 - DNA, 58 bp, Artificial Sequence
  Synthetic Sox17 ShRNA 2 sequence
ccggcgcacggaattcgaacagtatctcgagatactgttcgaattccgtgcgtttttg

SEQ ID NO: 61 - DNA, 58 bp, Artificial Sequence
  Synthetic Ezh2 ShRNA 1 sequence
ccgggctaggctaattgggaccaaactcgagtttggtcccaattagcctagctttttg

SEQ ID NO: 62 - DNA, 58 bp, Artificial Sequence
  Synthetic Ezh2 ShRNA 2 sequence
ccggcggctcctctaaccatgtttactcgagtaaacatggttagaggagccgtttttg

SEQ ID NO: 63 - DNA, 58 bp, Artificial Sequence
  Synthetic control ShRNA  sequence
ccggcaacaagatgaagagcaccaactcgagttggtgctcttcatcttgttgtttttg